European Patent Application EP 4 796 127 A1, published August 26, 2026. Title: 基于寡核苷酸的靶向降解Lin28A/B的PROTAC分子及其应用. Applicant: 北京大学. The sequence listing filed with the application follows.

SEQUENCE LISTING (24 sequences)

SEQ ID NO: 1 - RNA, 27 nt, synthetic construct
  source 1..27: mol_type = other RNA
ttagggtcacacccaccactgggagat

SEQ ID NO: 2 - RNA, 21 nt, synthetic construct
  source 1..21: mol_type = other RNA
ttagggtcacacccaccactg

SEQ ID NO: 3 - RNA, 21 nt, synthetic construct
  source 1..21: mol_type = other RNA
tagaattacatcaagggagat

SEQ ID NO: 4 - RNA, 15 nt, synthetic construct
  source 1..15: mol_type = other RNA
tagaattacatcaag

SEQ ID NO: 5 - RNA, 24 nt, Synthetic construct
  source 1..24: mol_type = other RNA
tggggctctgccctgctatgggat

SEQ ID NO: 6 - RNA, 18 nt, synthetic construct
  source 1..18: mol_type = other RNA
tggggctctgccctgcta

SEQ ID NO: 7 - RNA, 30 nt, synthetic construct
  source 1..30: mol_type = other RNA
tcagggcagtgatgttgcccctcggaagat

SEQ ID NO: 8 - RNA, 24 nt, synthetic construct
  source 1..24: mol_type = other RNA
tcagggcagtgatgttgcccctcg

SEQ ID NO: 9 - RNA, 21 nt, synthetic construct
  source 1..21: mol_type = other RNA
tagagttacaccctgggagtt

SEQ ID NO: 10 - RNA, 15 nt, synthetic construct
  source 1..15: mol_type = other RNA
tagagttacaccctg

SEQ ID NO: 11 - RNA, 30 nt, synthetic construct
  source 1..30: mol_type = other RNA
ttagggcagggattttgcccacaaggaggt

SEQ ID NO: 12 - RNA, 24 nt, synthetic construct
  source 1..24: mol_type = other RNA
ttagggcagggattttgcccacaa

SEQ ID NO: 13 - RNA, 21 nt, synthetic construct
  source 1..21: mol_type = other RNA
gaggaggacacccaaggagat

SEQ ID NO: 14 - RNA, 15 nt, synthetic construct
  source 1..15: mol_type = other RNA
gaggaggacacccaa

SEQ ID NO: 15 - RNA, 32 nt, synthetic construct
  source 1..32: mol_type = other RNA
gtggggtagtgattttaccctgttcaggagat

SEQ ID NO: 16 - RNA, 26 nt, synthetic construct
  source 1..26: mol_type = other RNA
gtggggtagtgattttaccctgttca

SEQ ID NO: 17 - RNA, 26 nt, synthetic construct
  source 1..26: mol_type = other RNA
ttagggtcataccccatcttggagat

SEQ ID NO: 18 - RNA, 20 nt, synthetic construct
  source 1..20: mol_type = other RNA
ttagggtcataccccatctt

SEQ ID NO: 19 - RNA, 33 nt, synthetic construct
  source 1..33: mol_type = other RNA
tgagggtctatgataccacccggtacaggagat

SEQ ID NO: 20 - RNA, 27 nt, synthetic construct
  source 1..27: mol_type = other RNA
tgagggtctatgataccacccggtaca

SEQ ID NO: 21 - RNA, 32 nt, synthetic construct
  source 1..32: mol_type = other RNA
ggtcgggttgtgacattgcccgctgtggagat

SEQ ID NO: 22 - RNA, 26 nt, synthetic construct
  source 1..26: mol_type = other RNA
ggtcgggttgtgacattgcccgctgt

SEQ ID NO: 23 - RNA, 34 nt, synthetic construct
  source 1..34: mol_type = other RNA
gtggggtagggatattaggccccaattagaagat

SEQ ID NO: 24 - RNA, 27 nt, synthetic construct
  source 1..27: mol_type = other RNA
gtggggtagggatattaggccccaatt